European Patent Specification EP 3 069 732 B1, published July 12, 2023. Title: Corneal Endothelial Therapeutics by promoting cell growth or inhibiting cell disorder. Applicant: THE DOSHISHA. The sequence listing filed with the application follows.

SEQUENCE LISTING (4 sequences)

SEQ ID NO: 1 - DNA, 22 bp, Artificial
  IL6-F primer
cacaagcgccttcggtccagtt

SEQ ID NO: 2 - DNA, 22 bp, Artificial
  IL6-R primer
tctgccagtgcctctttgctgc

SEQ ID NO: 3 - DNA, 20 bp, Artificial
  GAPDH-F
gagtcaacggatttggtcgt

SEQ ID NO: 4 - DNA, 20 bp, Artificial
  GAPDH-R
ttgattttggagggatctcg